European Patent Specification EP 3 419 414 B1, published August 13, 2025. Title: POWDERY MILDEW RESISTANCE GENES IN CARROT. Applicant: Bejo Zaden BV. The sequence listing filed with the application follows.

SEQUENCE LISTING (30 sequences)

SEQ ID NO: 1 - DNA, 101 bp, Daucus carota
ctgacccgacccgagactcgccgacctcttcaactccctccctccagacatcacccgacccgacccgccgtcaaacccgacaaaatcctcctccgacatcg

SEQ ID NO: 2 - DNA, 101 bp, Daucus carota
aatcttgaagttagtagcctttattggccttatgcttggcaacatcctgcggagacaaataggactatgtacaatagcagcagaattgcagtttttgataa

SEQ ID NO: 3 - DNA, 101 bp, Daucus carota
ttctcaaaaattcggaagaaaatgcaaatgcttaccwgggcacaagatgaccgttccaacggattggtcttatggatgtgagccagattttaagccttcag

SEQ ID NO: 4 - DNA, 101 bp, Daucus carota
ggtaatgtacttaaaaaaaagcactccaacactcttctagtggttacttagatcaccagcayawyctcaaatytcctagccattacctatttataagtaac

SEQ ID NO: 5 - DNA, 101 bp, Daucus carota
gcctttgcactcgagggccgatctcagtccggtctgaggaaatctttgcaggcctccgttagacctacgccccgtagaaactatcatcatgtccgcttgcc

SEQ ID NO: 6 - DNA, 101 bp, Daucus carota
cctaatgacagggctgaaatctgggcggtccgaaaggcaaacagagcaaccaccgactctcgtatatcctttcattcttcctgtccctccaatttttttaa

SEQ ID NO: 7 - DNA, 101 bp, Daucus carota
gatacttcagagtgctcaatgaacttggcaacggatcatcttcgaaggtttcttcgagaaccaaaccaattaagtgactggggtaaggcaccaagtccttg

SEQ ID NO: 8 - DNA, 101 bp, Daucus carota
taataacgtatatatatatgatatgacttctagcacttggttgaaagataaaaatcattgaaacacttggtttgaacccttcgattgaagataaggtctct

SEQ ID NO: 9 - DNA, 101 bp, Daucus carota
gccattagaggaaccaataactgtgaacaggcgcggcttaagtaaataacttttatagctgggacagactagtcgagtaatgtctatcaaaaccgatggtt

SEQ ID NO: 10 - DNA, 101 bp, Daucus carota
ttgaattctgctgtaaacttggtcatgtcctcctggtgatggcactattataattaacatggacggggctctgtttcattaaaagcagagttaatagtttc

SEQ ID NO: 11 - DNA, 101 bp, Daucus carota
tacgtctgtagtatgagtgtkttttcatgaattcggggtctgagataatacatcgccacgacttgcagaccaagctactcctcatcagtgatttagcagga

SEQ ID NO: 12 - DNA, 101 bp, Daucus carota
ctctaataccatttgtgttctaatatttcttgttcaggtcactttacttttacatcctaggtctggtgacccgtttctaagcttatctagtgatggttgtt

SEQ ID NO: 13 - DNA, 71 bp, Daucus carota
atccctgtcagaaaattgttacgtcggaaaagaaggcctcacgacgcgatcggaggagctgtagtaagagt

SEQ ID NO: 14 - DNA, 101 bp, Daucus carota
gcaagtattacccaaaattggccccaatatatattttttgtatccggctatattgattgcaccaatgtcacaatcttgaccawgaaaaaagactcccttaa

SEQ ID NO: 15 - DNA, 101 bp, Daucus carota
tgtacgatatatgttcagtctgttcttgagcctgattttacacaatctttgaatccgcgctggaaaaatgaaactttagaaggttttctttgatctcttaa

SEQ ID NO: 16 - DNA, 101 bp, Daucus carota
ctgacccgacccgagactcgccgacctcttcaactccctccctccagacaccacccgacccgacccgccgtcaaacccgacaaaatcctcctccgacatcg

SEQ ID NO: 17 - DNA, 101 bp, Daucus carota
aatcttgaagttagtagcctttattggccttatgcttggcaacatcctgcagagacaaataggactatgtacaatagcagcagaattgcagtttttgataa

SEQ ID NO: 18 - DNA, 101 bp, Daucus carota
ttctcaaaaattcggaagaaaatgcaaatgcttaccwgggcacaagatgaacgttccaacggattggtcttatggatgtgagccagattttaagccttcag

SEQ ID NO: 19 - DNA, 101 bp, Daucus carota
ggtaatgtacttaaaaaaaagcactccaacactcttctagtggttacttaaatcaccagcayawyctcaaatytcctagccattacctatttataagtaac

SEQ ID NO: 20 - DNA, 101 bp, Daucus carota
gcctttgcactcgagggccgatctcagtccggtctgaggaaatctttgcacgcctccgttagacctacgccccgtagaaactatcatcatgtccgcttgcc

SEQ ID NO: 21 - DNA, 101 bp, Daucus carota
cctaatgacagggctgaaatctgggcggtccgaaaggcaaacagagcaactaccgactctcgtatatcctttcattcttcctgtccctccaatttttttaa

SEQ ID NO: 22 - DNA, 101 bp, Daucus carota
gatacttcagagtgctcaatgaacttggcaacggatcatcttcgaaggttccttcgagaaccaaaccaattaagtgactggggtaaggcaccaagtccttg

SEQ ID NO: 23 - DNA, 101 bp, Daucus carota
taataacgtatatatatatgatatgacttctagcacttggttgaaagatagaaatcattgaaacacttggtttgaacccttcgattgaagataaggtctct

SEQ ID NO: 24 - DNA, 101 bp, Daucus carota
gccattagaggaaccaataactgtgaacaggcgcggcttaagtaaataacatttatagctgggacagactagtcgagtaatgtctatcaaaaccgatggtt

SEQ ID NO: 25 - DNA, 101 bp, Daucus carota
ttgaattctgctgtaaacttggtcatgtcctcctggtgatggcactattaaaattaacatggacggggctctgtttcattaaaagcagagttaatagtttc

SEQ ID NO: 26 - DNA, 101 bp, Daucus carota
tacgtctgtagtatgagtgtkttttcatgaattcggggtctgagataatagatcgccacgacttgcagaccaagctactcctcatcagtgatttagcagga

SEQ ID NO: 27 - DNA, 101 bp, Daucus carota
ctctaataccatttgtgttctaatatttcttgttcaggtcactttactttgacatcctaggtctggtgacccgtttctaagcttatctagtgatggttgtt

SEQ ID NO: 28 - DNA, 71 bp, Daucus carota
atccctgtcagaaaattgttacgtcggaaaagaaggcttcacgacgcgatcggaggagctgtagtaagagt

SEQ ID NO: 29 - DNA, 101 bp, Daucus carota
gcaagtattacccaaaattggccccaatatatattttttgtatccggctacattgattgcaccaatgtcacaatcttgaccawgaaaaaagactcccttaa

SEQ ID NO: 30 - DNA, 101 bp, Daucus carota
tgtacgatatatgttcagtctgttcttgagcctgattttacacaatctttaaatccgcgctggaaaaatgaaactttagaaggttttctttgatctcttaa